European Patent Application EP 4 610 361 A1, published September 3, 2025. Title: Extracellular vesicles overexpressed fiobronectin fragment protein and use for drug delivery thereof. Applicant: Dongguk University Industry-Academic Cooperation Foundation. The sequence listing filed with the application follows.

SEQUENCE LISTING (3 sequences)

SEQ ID NO: 1 - protein, 271 aa, synthetic construct
VPRDLEVVAATPTSLLISWDAPAVTVRYYRITYGETGGNSPVQEFTVPGSKSTATISGLKPGVDYTITVYAVTGRGDSPASSKPISINYRTEIDKPSQMQVTDVQDNSISVKWLPSSSPVTGYRVTTTPKNGPGPTKTKTAGPDQTEMTIEGLQPTVEYVVSVYAQNPSGESQPLVQTAVTNIDRPKGLAFTDVDVDSIKIAWESPQGQVSRYRVTYSSPEDGIHELFPAPDGEEDTAELQGLRPGSEYTVSVVALHDDMESQPLIGTQST

SEQ ID NO: 2 - protein, 275 aa, synthetic construct
AIPAPTDLKFTQVTPTSLSAQWTPPNVQLTGYRVRVTPKEKTGPMKEINLAPDSSSVVVSGLMVATKYEVSVYALKDTLTSRPAQGVVTTLENVSPPRRARVTDATETTITISWRTKTETITGFQVDAVPANGQTPIQRTIKPDVRSYTITGLQPGTDYKIYLYTLNDNARSSPVVIDASTAIDAPSNLRFLATTPNSLLVSWQPPRARITGYIIKYEKPGSPPREVVPRPRPGVTEATITGLEPGTEYTIYVIALKNNQKSEPLIGRKKTDELP

SEQ ID NO: 3 - protein, 382 aa, synthetic construct [sequence omitted]